European Patent Application EP 4 393 949 A1, published July 3, 2024. Title: PHARMACEUTICAL COMPOSITION CONTAINING FUSION PROTEIN. Applicant: JIANGSU HENGRUI PHARMACEUTICALS CO., LTD. Application CN. The sequence listing filed with the application follows.

SEQUENCE LISTING (190 sequences)

SEQ ID NO: 1 - protein, 123 aa, Artificial Sequence
  DOMAIN 1..123: note = A2-22 VH
QVQLVQSGAEVKKPGASVKVSCKASGYTFTSYYMHWVRQAPGQGLEWMGIINPSGGSTSYAQKFQGRVTMTRDTSTSTVYMELSSLRSEDTAVYYCAREDWMEYEYYYGMDVWGQGTLVTVSS

SEQ ID NO: 2 - protein, 108 aa, Artificial Sequence
  DOMAIN 1..108: note = A2-22 VL
EIVLTQSPGTLSLSPGERATLSCRASQSVSNNYLAWYQQKPGQAPRLLIYGASSRATGIPDRFSGSGSGTDFTLTISRLEPEDFAVYSCQQYGSSPLTFGQGTRLEIK

SEQ ID NO: 3 - protein, 120 aa, Artificial Sequence
  DOMAIN 1..120: note = A3-21 VH
EVQLLESGGGLAQPGGSLRLSCAGSGFTFSSYAMSWVRQAPGKGLEWVSGITGTGYRTYYADSVKGRFTVSRDNSRNTVYLQMNSLRAEDTAVYYCVRESGHYYGWFDSWGQGTLVTVSS

SEQ ID NO: 4 - protein, 112 aa, Artificial Sequence
  DOMAIN 1..112: note = A3-21 VL
QSALTQPPSVSGAPGQRVTISCTGSSSNIGAGYNVHWYQQVPGTVPKLLIDGKGNRPSGVPDRFSGSKSGTSASLAITGLQAEDEADYYCQSYDYMLSGSVVFGRGTKLTVL

SEQ ID NO: 5 - protein, 122 aa, Artificial Sequence
  DOMAIN 1..122: note = B2-15 VH
EVQLLESGAEVKKPGASVKVSCKASGYTFTSYYMHWVRQAPGQGLEWMGIINPSGGSTSYAQKFQGRVTMTRDTSTSTVYMELSSLRSEDTAVYYCAREGNSSGYYNAFDIWGQGTMVTVSS

SEQ ID NO: 6 - protein, 108 aa, Artificial Sequence
  DOMAIN 1..108: note = B2-15 VL
EIVLTQSPGTLSLSPGERATLSCRASQSVSSSYLAWYQQKPGQAPRLLIYGASNRATGIPDRFSGSGSGADFTLTISRLEPEDFAVYYCQQYGSSPLTFGGGTKVEIK

SEQ ID NO: 7 - protein, 124 aa, Artificial Sequence
  DOMAIN 1..124: note = C2-53 VH
EVQLVESGGGLVQPGRSLILSCAASGFTFDDYAMHWVRQAPGKGLEWVSGISWNSGSIGYADSVKGRFTISRDNAKNSLYLQMNSLRAEDTALYYCAKDQLRWGTYYYYGMDVWGQGTTVTVSS

SEQ ID NO: 8 - protein, 106 aa, Artificial Sequence
  DOMAIN 1..106: note = C2-53 VL
DIQMTQSPSTLSASVGDRVTITCRASQSVSIWVAWYQQKPGKAPKLLIYKASSLERGVPTRFSGSGSGTEFTLTISSLQPEDFATYHCQQYDTGATFGQGTKVEMK

SEQ ID NO: 9 - protein, 121 aa, Artificial Sequence
  DOMAIN 1..121: note = D2-60 VH
QVQLVQSGAEVKKPGASVKVSCKASGYTFTSYGISWVRQAPGQGLEWMGWISAYNGNTNYAQKLQGRVTMTTDTSTSTAYMELRSLRSDDTAVYYCAREYSSWYSGGMDVWGQGTTVTVSS

SEQ ID NO: 10 - protein, 107 aa, Artificial Sequence
  DOMAIN 1..107: note = D2-60 VL
DIQMTQSPSSLSASVGDRVTITCRASQGISNYLAWYQQKPGKVPKLLIYAASTLQSGVPSRFSGSGSGTDFTLTISSLQPEDVATYYCQKYDSAPFTFGQGTRLEIK

SEQ ID NO: 11 - protein, 125 aa, Artificial Sequence
  DOMAIN 1..125: note = D3-68 VH
QVQLVQSGPEVKKPGASVKVSCKASGYTFTSYGISWVRRAPGQGLEWMGWISAYNGNTNYAQKLQGRVTMTTDTSTSTAYMELRSLRSDDTAVYYCARDLQSPTYYYGSGVIDYWGQGTLVTVSS

SEQ ID NO: 12 - protein, 107 aa, Artificial Sequence
  DOMAIN 1..107: note = D3-68 VL
DIQLTQSPSTLSASVGDRVTISCRASRAVSPWLAWYQHRPGQAPKLLIYAASSLQSGVPSRFSGSGSGTDFTLTISSLQPEDFATYYCQQYRSYPFTFGPGTTVDIR

SEQ ID NO: 13 - protein, 5 aa, Artificial Sequence
  DOMAIN 1..5: note = A2-22 HCDR1 kabat
SYYMH

SEQ ID NO: 14 - protein, 17 aa, Artificial Sequence
  DOMAIN 1..17: note = A2-22 HCDR2 kabat
IINPSGGSTSYAQKFQG

SEQ ID NO: 15 - protein, 14 aa, Artificial Sequence
  DOMAIN 1..14: note = A2-22 HCDR3 kabat
EDWMEYEYYYGMDV

SEQ ID NO: 16 - protein, 12 aa, Artificial Sequence
  DOMAIN 1..12: note = A2-22 LCDR1 kabat
RASQSVSNNYLA

SEQ ID NO: 17 - protein, 7 aa, Artificial Sequence
  DOMAIN 1..7: note = A2-22 LCDR2 kabat
GASSRAT

SEQ ID NO: 18 - protein, 9 aa, Artificial Sequence
  DOMAIN 1..9: note = A2-22 LCDR3 kabat
QQYGSSPLT

SEQ ID NO: 19 - protein, 5 aa, Artificial Sequence
  DOMAIN 1..5: note = A3-21 HCDR1 kabat
SYAMS

SEQ ID NO: 20 - protein, 17 aa, Artificial Sequence
  DOMAIN 1..17: note = A3-21 HCDR2 kabat
GITGTGYRTYYADSVKG

SEQ ID NO: 21 - protein, 11 aa, Artificial Sequence
  DOMAIN 1..11: note = A3-21 HCDR3 kabta
ESGHYYGWFDS

SEQ ID NO: 22 - protein, 14 aa, Artificial Sequence
  DOMAIN 1..14: note = A3-21 LCDR1 kabat
TGSSSNIGAGYNVH

SEQ ID NO: 23 - protein, 7 aa, Artificial Sequence
  DOMAIN 1..7: note = A3-21 LCDR2 kabat
GKGNRPS

SEQ ID NO: 24 - protein, 12 aa, Artificial Sequence
  DOMAIN 1..12: note = A3-21 LCDR3 kabat
QSYDYMLSGSVV

SEQ ID NO: 25 - protein, 5 aa, Artificial Sequence
  DOMAIN 1..5: note = B2-15 HCDR1 kabat
SYYMH

SEQ ID NO: 26 - protein, 17 aa, Artificial Sequence
  DOMAIN 1..17: note = B2-15 HCDR2 kabat
IINPSGGSTSYAQKFQG

SEQ ID NO: 27 - protein, 13 aa, Artificial Sequence
  DOMAIN 1..13: note = B2-15 HCDR3 kabat
EGNSSGYYNAFDI

SEQ ID NO: 28 - protein, 12 aa, Artificial Sequence
  DOMAIN 1..12: note = B2-15 LCDR1 kabat
RASQSVSSSYLA

SEQ ID NO: 29 - protein, 7 aa, Artificial Sequence
  DOMAIN 1..7: note = B2-15 LCDR2 kabat
GASNRAT

SEQ ID NO: 30 - protein, 9 aa, Artificial Sequence
  DOMAIN 1..9: note = B2-15 LCDR3 kabat
QQYGSSPLT

SEQ ID NO: 31 - protein, 5 aa, Artificial Sequence
  DOMAIN 1..5: note = C2-53 HCDR1 kabat
DYAMH

SEQ ID NO: 32 - protein, 17 aa, Artificial Sequence
  DOMAIN 1..17: note = C2-53 HCDR2 kabat
GISWNSGSIGYADSVKG

SEQ ID NO: 33 - protein, 15 aa, Artificial Sequence
  DOMAIN 1..15: note = C2-53 HCDR3 kabat
DQLRWGTYYYYGMDV

SEQ ID NO: 34 - protein, 11 aa, Artificial Sequence
  DOMAIN 1..11: note = C2-53 LCDR1 kabat
RASQSVSIWVA

SEQ ID NO: 35 - protein, 7 aa, Artificial Sequence
  DOMAIN 1..7: note = C2-53 LCDR2 kabat
KASSLER

SEQ ID NO: 36 - protein, 8 aa, Artificial Sequence
  DOMAIN 1..8: note = C2-53 LCDR3 kabat
QQYDTGAT

SEQ ID NO: 37 - protein, 5 aa, Artificial Sequence
  DOMAIN 1..5: note = D2-60 HCDR1 kabat
SYGIS

SEQ ID NO: 38 - protein, 17 aa, Artificial Sequence
  DOMAIN 1..17: note = D2-60 HCDR2 kabat
WISAYNGNTNYAQKLQG

SEQ ID NO: 39 - protein, 12 aa, Artificial Sequence
  DOMAIN 1..12: note = D2-60 HCDR3 kabat
EYSSWYSGGMDV

SEQ ID NO: 40 - protein, 11 aa, Artificial Sequence
  DOMAIN 1..11: note = D2-60 LCDR1 kabat
RASQGISNYLA

SEQ ID NO: 41 - protein, 7 aa, Artificial Sequence
  DOMAIN 1..7: note = D2-60 LCDR2 kabat
AASTLQS

SEQ ID NO: 42 - protein, 9 aa, Artificial Sequence
  DOMAIN 1..9: note = D2-60 LCDR3 kabat
QKYDSAPFT

SEQ ID NO: 43 - protein, 5 aa, Artificial Sequence
  DOMAIN 1..5: note = D3-68 HCDR1 kabat
SYGIS

SEQ ID NO: 44 - protein, 17 aa, Artificial Sequence
  DOMAIN 1..17: note = D3-68 HCDR2 kabat
WISAYNGNTNYAQKLQG

SEQ ID NO: 45 - protein, 16 aa, Artificial Sequence
  DOMAIN 1..16: note = D3-68 HCDR3 kabat
DLQSPTYYYGSGVIDY

SEQ ID NO: 46 - protein, 11 aa, Artificial Sequence
  DOMAIN 1..11: note = D3-68 LCDR1 kabat
RASRAVSPWLA

SEQ ID NO: 47 - protein, 7 aa, Artificial Sequence
  DOMAIN 1..7: note = D3-68 LCDR2 kabat
AASSLQS

SEQ ID NO: 48 - protein, 9 aa, Artificial Sequence
  DOMAIN 1..9: note = D3-68 LCDR3 kabat
QQYRSYPFT

SEQ ID NO: 49 - protein, 7 aa, Artificial Sequence
  DOMAIN 1..7: note = A2-22 HCDR1 cho
GYTFTSY

SEQ ID NO: 50 - protein, 6 aa, Artificial Sequence
  DOMAIN 1..6: note = A2-22 HCDR2 cho
NPSGGS

SEQ ID NO: 51 - protein, 14 aa, Artificial Sequence
  DOMAIN 1..14: note = A2-22 HCDR3 cho
EDWMEYEYYYGMDV

SEQ ID NO: 52 - protein, 12 aa, Artificial Sequence
  DOMAIN 1..12: note = A2-22 LCDR1 cho
RASQSVSNNYLA

SEQ ID NO: 53 - protein, 7 aa, Artificial Sequence
  DOMAIN 1..7: note = A2-22 LCDR2 cho
GASSRAT

SEQ ID NO: 54 - protein, 9 aa, Artificial Sequence
  DOMAIN 1..9: note = A2-22 LCDR3 cho
QQYGSSPLT

SEQ ID NO: 55 - protein, 7 aa, Artificial Sequence
  DOMAIN 1..7: note = A3-21 HCDR1 cho
GFTFSSY

SEQ ID NO: 56 - protein, 6 aa, Artificial Sequence
  DOMAIN 1..6: note = A3-21 HCDR2 cho
TGTGYR

SEQ ID NO: 57 - protein, 11 aa, Artificial Sequence
  DOMAIN 1..11: note = A3-21 HCDR3 cho
ESGHYYGWFDS

SEQ ID NO: 58 - protein, 14 aa, Artificial Sequence
  DOMAIN 1..14: note = A3-21 LCDR1 cho
TGSSSNIGAGYNVH

SEQ ID NO: 59 - protein, 7 aa, Artificial Sequence
  DOMAIN 1..7: note = A3-21 LCDR2 cho
GKGNRPS

SEQ ID NO: 60 - protein, 12 aa, Artificial Sequence
  DOMAIN 1..12: note = A3-21 LCDR3 cho
QSYDYMLSGSVV

SEQ ID NO: 61 - protein, 7 aa, Artificial Sequence
  DOMAIN 1..7: note = B2-15 HCDR1 cho
GYTFTSY

SEQ ID NO: 62 - protein, 6 aa, Artificial Sequence
  DOMAIN 1..6: note = B2-15 HCDR2 cho
NPSGGS

SEQ ID NO: 63 - protein, 13 aa, Artificial Sequence
  DOMAIN 1..13: note = B2-15 HCDR3 cho
EGNSSGYYNAFDI

SEQ ID NO: 64 - protein, 12 aa, Artificial Sequence
  DOMAIN 1..12: note = B2-15 LCDR1 cho
RASQSVSSSYLA

SEQ ID NO: 65 - protein, 7 aa, Artificial Sequence
  DOMAIN 1..7: note = B2-15 LCDR2 cho
GASNRAT

SEQ ID NO: 66 - protein, 9 aa, Artificial Sequence
  DOMAIN 1..9: note = B2-15 LCDR3 cho
QQYGSSPLT

SEQ ID NO: 67 - protein, 7 aa, Artificial Sequence
  DOMAIN 1..7: note = C2-53 HCDR1 cho
GFTFDDY

SEQ ID NO: 68 - protein, 6 aa, Artificial Sequence
  DOMAIN 1..6: note = C2-53 HCDR2 cho
SWNSGS

SEQ ID NO: 69 - protein, 15 aa, Artificial Sequence
  DOMAIN 1..15: note = C3-53 HCDR3 cho
DQLRWGTYYYYGMDV

SEQ ID NO: 70 - protein, 11 aa, Artificial Sequence
  DOMAIN 1..11: note = C2-53 LCDR1 cho
RASQSVSIWVA

SEQ ID NO: 71 - protein, 7 aa, Artificial Sequence
  DOMAIN 1..7: note = C2-53 LCDR2 cho
KASSLER

SEQ ID NO: 72 - protein, 8 aa, Artificial Sequence
  DOMAIN 1..8: note = C2-53 LCDR3 cho
QQYDTGAT

SEQ ID NO: 73 - protein, 7 aa, Artificial Sequence
  DOMAIN 1..7: note = D2-60 HCDR1 cho
GYTFTSY

SEQ ID NO: 74 - protein, 6 aa, Artificial Sequence
  DOMAIN 1..6: note = D2-60 HCDR2 cho
SAYNGN

SEQ ID NO: 75 - protein, 12 aa, Artificial Sequence
  DOMAIN 1..12: note = D2-60 HCDR3 cho
EYSSWYSGGMDV

SEQ ID NO: 76 - protein, 11 aa, Artificial Sequence
  DOMAIN 1..11: note = D2-60 LCDR1 cho
RASQGISNYLA

SEQ ID NO: 77 - protein, 7 aa, Artificial Sequence
  DOMAIN 1..7: note = D2-60 LCDR2 cho
AASTLQS

SEQ ID NO: 78 - protein, 9 aa, Artificial Sequence
  DOMAIN 1..9: note = D2-69 LCDR3 cho
QKYDSAPFT

SEQ ID NO: 79 - protein, 7 aa, Artificial Sequence
  DOMAIN 1..7: note = D3-68 HCDR1 cho
GYTFTSY

SEQ ID NO: 80 - protein, 6 aa, Artificial Sequence
  DOMAIN 1..6: note = D3-68 HCDR2 cho
SAYNGN

SEQ ID NO: 81 - protein, 16 aa, Artificial Sequence
  DOMAIN 1..16: note = D3-68 HCDR3 cho
DLQSPTYYYGSGVIDY

SEQ ID NO: 82 - protein, 11 aa, Artificial Sequence
  DOMAIN 1..11: note = D3-68 LCDR1 cho
RASRAVSPWLA

SEQ ID NO: 83 - protein, 7 aa, Artificial Sequence
  DOMAIN 1..7: note = D3-68 LCDR2 cho
AASSLQS

SEQ ID NO: 84 - protein, 9 aa, Artificial Sequence
  DOMAIN 1..9: note = D3-68 LCDR3 cho
QQYRSYPFT

SEQ ID NO: 85 - protein, 8 aa, Artificial Sequence
  DOMAIN 1..8: note = A2-22 HCDR1 IMGT
GYTFTSYY

SEQ ID NO: 86 - protein, 8 aa, Artificial Sequence
  DOMAIN 1..8: note = A2-22 HCDR2 IMGT
INPSGGST

SEQ ID NO: 87 - protein, 16 aa, Artificial Sequence
  DOMAIN 1..16: note = A2-22 HCDR3 IMGT
AREDWMEYEYYYGMDV

SEQ ID NO: 88 - protein, 7 aa, Artificial Sequence
  DOMAIN 1..7: note = A2-22 LCDR1 IMGT
QSVSNNY

SEQ ID NO: 89 - skipped

SEQ ID NO: 90 - protein, 9 aa, Artificial Sequence
  DOMAIN 1..9: note = A2-22 LCDR3 IMGT
QQYGSSPLT

SEQ ID NO: 91 - protein, 8 aa, Artificial Sequence
  DOMAIN 1..8: note = A3-21 HCDR1 IMGT
GFTFSSYA

SEQ ID NO: 92 - protein, 8 aa, Artificial Sequence
  DOMAIN 1..8: note = A3-21 HCDR2 IMGT
ITGTGYRT

SEQ ID NO: 93 - protein, 13 aa, Artificial Sequence
  DOMAIN 1..13: note = A3-21 HCDR3 IMGT
VRESGHYYGWFDS

SEQ ID NO: 94 - protein, 9 aa, Artificial Sequence
  DOMAIN 1..9: note = A3-21 LCDR1 IMGT
SSNIGAGYN

SEQ ID NO: 95 - skipped

SEQ ID NO: 96 - protein, 12 aa, Artificial Sequence
  DOMAIN 1..12: note = A3-21 LCDR3 IMGT
QSYDYMLSGSVV

SEQ ID NO: 97 - protein, 8 aa, Artificial Sequence
  DOMAIN 1..8: note = B2-15 HCDR1 IMGT
GYTFTSYY

SEQ ID NO: 98 - protein, 8 aa, Artificial Sequence
  DOMAIN 1..8: note = B2-15 HCDR2 IMGT
INPSGGST

SEQ ID NO: 99 - protein, 15 aa, Artificial Sequence
  DOMAIN 1..15: note = B2-15 HCDR3 IMGT
AREGNSSGYYNAFDI

SEQ ID NO: 100 - protein, 7 aa, Artificial Sequence
  DOMAIN 1..7: note = B2-15 LCDR1 IMGT
QSVSSSY

SEQ ID NO: 101 - skipped

SEQ ID NO: 102 - protein, 9 aa, Artificial Sequence
  DOMAIN 1..9: note = B2-15 LCDR3 IMGT
QQYGSSPLT

SEQ ID NO: 103 - protein, 8 aa, Artificial Sequence
  DOMAIN 1..8: note = C2-53 HCDR1 IMGT
GFTFDDYA

SEQ ID NO: 104 - protein, 8 aa, Artificial Sequence
  DOMAIN 1..8: note = C2-53 HCDR2 IMGT
ISWNSGSI

SEQ ID NO: 105 - protein, 17 aa, Artificial Sequence
  DOMAIN 1..17: note = C2-53 HCDR3 IMGT
AKDQLRWGTYYYYGMDV

SEQ ID NO: 106 - protein, 6 aa, Artificial Sequence
  DOMAIN 1..6: note = C2-53 LCDR1 IMGT
QSVSIW

SEQ ID NO: 107 - skipped

SEQ ID NO: 108 - protein, 8 aa, Artificial Sequence
  DOMAIN 1..8: note = C2-53 LCDR3 IMGT
QQYDTGAT

SEQ ID NO: 109 - protein, 8 aa, Artificial Sequence
  DOMAIN 1..8: note = D2-60 HCDR1 IMGT
GYTFTSYG

SEQ ID NO: 110 - protein, 8 aa, Artificial Sequence
  DOMAIN 1..8: note = D2-60 HCDR2 IMGT
ISAYNGNT

SEQ ID NO: 111 - protein, 14 aa, Artificial Sequence
  DOMAIN 1..14: note = D2-60 HCDR3 IMGT
AREYSSWYSGGMDV

SEQ ID NO: 112 - protein, 6 aa, Artificial Sequence
  DOMAIN 1..6: note = D2-60 LCDR1 IMGT
QGISNY

SEQ ID NO: 113 - skipped

SEQ ID NO: 114 - protein, 9 aa, Artificial Sequence
  DOMAIN 1..9: note = D2-60 LCDR3 IMGT
QKYDSAPFT

SEQ ID NO: 115 - protein, 8 aa, Artificial Sequence
  DOMAIN 1..8: note = D3-68 HCDR1 IMGT
GYTFTSYG

SEQ ID NO: 116 - protein, 8 aa, Artificial Sequence
  DOMAIN 1..8: note = D3-68 HCDR2 IMGT
ISAYNGNT

SEQ ID NO: 117 - protein, 18 aa, Artificial Sequence
  DOMAIN 1..18: note = D3-68 HCDR3 IMGT
ARDLQSPTYYYGSGVIDY

SEQ ID NO: 118 - protein, 6 aa, Artificial Sequence
  DOMAIN 1..6: note = D3-68 LCDR1 IMGT
RAVSPW

SEQ ID NO: 119 - skipped

SEQ ID NO: 120 - protein, 9 aa, Artificial Sequence
  DOMAIN 1..9: note = D3-68 LCDR3 IMGT
QQYRSYPFT

SEQ ID NO: 121 - protein, 10 aa, Artificial Sequence
  DOMAIN 1..10: note = A2-22 HCDR1 ABM
GYTFTSYYMH

SEQ ID NO: 122 - protein, 10 aa, Artificial Sequence
  DOMAIN 1..10: note = A2-22 HCDR2 ABM
IINPSGGSTS

SEQ ID NO: 123 - protein, 14 aa, Artificial Sequence
  DOMAIN 1..14: note = A2-22 HCDR3 ABM
EDWMEYEYYYGMDV

SEQ ID NO: 124 - protein, 12 aa, Artificial Sequence
  DOMAIN 1..12: note = A2-22 LCDR1 ABM
RASQSVSNNYLA

SEQ ID NO: 125 - protein, 7 aa, Artificial Sequence
  DOMAIN 1..7: note = A2-22 LCDR2 ABM
GASSRAT

SEQ ID NO: 126 - protein, 9 aa, Artificial Sequence
  DOMAIN 1..9: note = A2-22 LCDR3 ABM
QQYGSSPLT

SEQ ID NO: 127 - protein, 10 aa, Artificial Sequence
  DOMAIN 1..10: note = A3-21 HCDR1 ABM
GFTFSSYAMS

SEQ ID NO: 128 - protein, 10 aa, Artificial Sequence
  DOMAIN 1..10: note = A3-21 HCDR2 ABM
GITGTGYRTY

SEQ ID NO: 129 - protein, 11 aa, Artificial Sequence
  DOMAIN 1..11: note = A3-21 HCDR3 ABM
ESGHYYGWFDS

SEQ ID NO: 130 - protein, 14 aa, Artificial Sequence
  DOMAIN 1..14: note = A3-21 LCDR1 ABM
TGSSSNIGAGYNVH

SEQ ID NO: 131 - protein, 7 aa, Artificial Sequence
  DOMAIN 1..7: note = A3-21 LCDR2 ABM
GKGNRPS

SEQ ID NO: 132 - protein, 12 aa, Artificial Sequence
  DOMAIN 1..12: note = A3-21 LCDR3 ABM
QSYDYMLSGSVV

SEQ ID NO: 133 - protein, 10 aa, Artificial Sequence
  DOMAIN 1..10: note = B2-15 HCDR1 ABM
GYTFTSYYMH

SEQ ID NO: 134 - protein, 10 aa, Artificial Sequence
  DOMAIN 1..10: note = B2-15 HCDR2 ABM
IINPSGGSTS

SEQ ID NO: 135 - protein, 13 aa, Artificial Sequence
  DOMAIN 1..13: note = B2-15 HCDR3 ABM
EGNSSGYYNAFDI

SEQ ID NO: 136 - protein, 12 aa, Artificial Sequence
  DOMAIN 1..12: note = B2-15 LCDR1 ABM
RASQSVSSSYLA

SEQ ID NO: 137 - protein, 7 aa, Artificial Sequence
  DOMAIN 1..7: note = B2-15 LCDR2 ABM
GASNRAT

SEQ ID NO: 138 - protein, 9 aa, Artificial Sequence
  DOMAIN 1..9: note = B2-15 LCDR3 ABM
QQYGSSPLT

SEQ ID NO: 139 - protein, 10 aa, Artificial Sequence
  DOMAIN 1..10: note = C2-53 HCDR1 ABM
GFTFDDYAMH

SEQ ID NO: 140 - protein, 10 aa, Artificial Sequence
  DOMAIN 1..10: note = C2-53 HCDR2 ABM
GISWNSGSIG

SEQ ID NO: 141 - protein, 15 aa, Artificial Sequence
  DOMAIN 1..15: note = C2-53 HCDR3 ABM
DQLRWGTYYYYGMDV

SEQ ID NO: 142 - protein, 11 aa, Artificial Sequence
  DOMAIN 1..11: note = C2-53 LCDR1 ABM
RASQSVSIWVA

SEQ ID NO: 143 - protein, 7 aa, Artificial Sequence
  DOMAIN 1..7: note = C2-53 LCDR2 ABM
KASSLER

SEQ ID NO: 144 - protein, 8 aa, Artificial Sequence
  DOMAIN 1..8: note = C2-53 LCDR3 ABM
QQYDTGAT

SEQ ID NO: 145 - protein, 10 aa, Artificial Sequence
  DOMAIN 1..10: note = D2-60 HCDR1 ABM
GYTFTSYGIS

SEQ ID NO: 146 - protein, 10 aa, Artificial Sequence
  DOMAIN 1..10: note = D2-60 HCDR2 ABM
WISAYNGNTN

SEQ ID NO: 147 - protein, 12 aa, Artificial Sequence
  DOMAIN 1..12: note = D2-60 HCDR3 ABM
EYSSWYSGGMDV

SEQ ID NO: 148 - protein, 11 aa, Artificial Sequence
  DOMAIN 1..11: note = D2-60 LCDR1 ABM
RASQGISNYLA

SEQ ID NO: 149 - protein, 7 aa, Artificial Sequence
  DOMAIN 1..7: note = D2-60 LCDR2 ABM
AASTLQS

SEQ ID NO: 150 - protein, 9 aa, Artificial Sequence
  DOMAIN 1..9: note = D2-60 LCDR3 ABM
QKYDSAPFT

SEQ ID NO: 151 - protein, 10 aa, Artificial Sequence
  DOMAIN 1..10: note = D3-68 HCDR1 ABM
GYTFTSYGIS

SEQ ID NO: 152 - protein, 10 aa, Artificial Sequence
  DOMAIN 1..10: note = D3-68 HCDR2 ABM
WISAYNGNTN

SEQ ID NO: 153 - protein, 16 aa, Artificial Sequence
  DOMAIN 1..16: note = D3-68 HCDR3 ABM
DLQSPTYYYGSGVIDY

SEQ ID NO: 154 - protein, 11 aa, Artificial Sequence
  DOMAIN 1..11: note = D3-68 LCDR1 ABM
RASRAVSPWLA

SEQ ID NO: 155 - protein, 7 aa, Artificial Sequence
  DOMAIN 1..7: note = D3-68 LCDR2 ABM
AASSLQS

SEQ ID NO: 156 - protein, 9 aa, Artificial Sequence
  DOMAIN 1..9: note = D3-68 LCDR3 ABM
QQYRSYPFT

SEQ ID NO: 157 - protein, 453 aa, Artificial Sequence
  DOMAIN 1..453: note = A2-22 HC
QVQLVQSGAEVKKPGASVKVSCKASGYTFTSYYMHWVRQAPGQGLEWMGIINPSGGSTSYAQKFQGRVTMTRDTSTSTVYMELSSLRSEDTAVYYCAREDWMEYEYYYGMDVWGQGTLVTVSSASTKGPSVFPLAPSSKSTSGGTAALGCLVKDYFPEPVTVSWNSGALTSGVHTFPAVLQSSGLYSLSSVVTVPSSSLGTQTYICNVNHKPSNTKVDKKVEPKSCDKTHTCPPCPAPEAAGGPSVFLFPPKPKDTLMISRTPEVTCVVVDVSHEDPEVKFNWYVDGVEVHNAKTKPREEQYNSTYRVVSVLTVLHQDWLNGKEYKCKVSNKALPAPIEKTISKAKGQPREPQVYTLPPSRDELTKNQVSLTCLVKGFYPSDIAVEWESNGQPENNYKTTPPVLDSDGSFFLYSKLTVDKSRWQQGNVFSCSVMHEALHNHYTQKSLSLSPGK

SEQ ID NO: 158 - protein, 215 aa, Artificial Sequence
  DOMAIN 1..215: note = A2-22 LC
EIVLTQSPGTLSLSPGERATLSCRASQSVSNNYLAWYQQKPGQAPRLLIYGASSRATGIPDRFSGSGSGTDFTLTISRLEPEDFAVYSCQQYGSSPLTFGQGTRLEIKRTVAAPSVFIFPPSDEQLKSGTASVVCLLNNFYPREAKVQWKVDNALQSGNSQESVTEQDSKDSTYSLSSTLTLSKADYEKHKVYACEVTHQGLSSPVTKSFNRGEC

SEQ ID NO: 159 - protein, 450 aa, Artificial Sequence
  DOMAIN 1..450: note = A3-21 HC
EVQLLESGGGLAQPGGSLRLSCAGSGFTFSSYAMSWVRQAPGKGLEWVSGITGTGYRTYYADSVKGRFTVSRDNSRNTVYLQMNSLRAEDTAVYYCVRESGHYYGWFDSWGQGTLVTVSSASTKGPSVFPLAPSSKSTSGGTAALGCLVKDYFPEPVTVSWNSGALTSGVHTFPAVLQSSGLYSLSSVVTVPSSSLGTQTYICNVNHKPSNTKVDKKVEPKSCDKTHTCPPCPAPEAAGGPSVFLFPPKPKDTLMISRTPEVTCVVVDVSHEDPEVKFNWYVDGVEVHNAKTKPREEQYNSTYRVVSVLTVLHQDWLNGKEYKCKVSNKALPAPIEKTISKAKGQPREPQVYTLPPSRDELTKNQVSLTCLVKGFYPSDIAVEWESNGQPENNYKTTPPVLDSDGSFFLYSKLTVDKSRWQQGNVFSCSVMHEALHNHYTQKSLSLSPGK

SEQ ID NO: 160 - protein, 218 aa, Artificial Sequence
  DOMAIN 1..218: note = A3-21 LC
QSALTQPPSVSGAPGQRVTISCTGSSSNIGAGYNVHWYQQVPGTVPKLLIDGKGNRPSGVPDRFSGSKSGTSASLAITGLQAEDEADYYCQSYDYMLSGSVVFGRGTKLTVLGQPKANPTVTLFPPSSEELQANKATLVCLISDFYPGAVTVAWKADGSPVKAGVETTKPSKQSNNKYAASSYLSLTPEQWKSHRSYSCQVTHEGSTVEKTVAPTECS

SEQ ID NO: 161 - protein, 452 aa, Artificial Sequence
  DOMAIN 1..452: note = B2-15 HC
EVQLLESGAEVKKPGASVKVSCKASGYTFTSYYMHWVRQAPGQGLEWMGIINPSGGSTSYAQKFQGRVTMTRDTSTSTVYMELSSLRSEDTAVYYCAREGNSSGYYNAFDIWGQGTMVTVSSASTKGPSVFPLAPSSKSTSGGTAALGCLVKDYFPEPVTVSWNSGALTSGVHTFPAVLQSSGLYSLSSVVTVPSSSLGTQTYICNVNHKPSNTKVDKKVEPKSCDKTHTCPPCPAPEAAGGPSVFLFPPKPKDTLMISRTPEVTCVVVDVSHEDPEVKFNWYVDGVEVHNAKTKPREEQYNSTYRVVSVLTVLHQDWLNGKEYKCKVSNKALPAPIEKTISKAKGQPREPQVYTLPPSRDELTKNQVSLTCLVKGFYPSDIAVEWESNGQPENNYKTTPPVLDSDGSFFLYSKLTVDKSRWQQGNVFSCSVMHEALHNHYTQKSLSLSPGK

SEQ ID NO: 162 - protein, 215 aa, Artificial Sequence
  DOMAIN 1..215: note = B2-15 LC
EIVLTQSPGTLSLSPGERATLSCRASQSVSSSYLAWYQQKPGQAPRLLIYGASNRATGIPDRFSGSGSGADFTLTISRLEPEDFAVYYCQQYGSSPLTFGGGTKVEIKRTVAAPSVFIFPPSDEQLKSGTASVVCLLNNFYPREAKVQWKVDNALQSGNSQESVTEQDSKDSTYSLSSTLTLSKADYEKHKVYACEVTHQGLSSPVTKSFNRGEC

SEQ ID NO: 163 - protein, 454 aa, Artificial Sequence
  DOMAIN 1..454: note = C2-53 HC
EVQLVESGGGLVQPGRSLILSCAASGFTFDDYAMHWVRQAPGKGLEWVSGISWNSGSIGYADSVKGRFTISRDNAKNSLYLQMNSLRAEDTALYYCAKDQLRWGTYYYYGMDVWGQGTTVTVSSASTKGPSVFPLAPSSKSTSGGTAALGCLVKDYFPEPVTVSWNSGALTSGVHTFPAVLQSSGLYSLSSVVTVPSSSLGTQTYICNVNHKPSNTKVDKKVEPKSCDKTHTCPPCPAPEAAGGPSVFLFPPKPKDTLMISRTPEVTCVVVDVSHEDPEVKFNWYVDGVEVHNAKTKPREEQYNSTYRVVSVLTVLHQDWLNGKEYKCKVSNKALPAPIEKTISKAKGQPREPQVYTLPPSRDELTKNQVSLTCLVKGFYPSDIAVEWESNGQPENNYKTTPPVLDSDGSFFLYSKLTVDKSRWQQGNVFSCSVMHEALHNHYTQKSLSLSPGK

SEQ ID NO: 164 - protein, 213 aa, Artificial Sequence
  DOMAIN 1..213: note = C2-53 LC
DIQMTQSPSTLSASVGDRVTITCRASQSVSIWVAWYQQKPGKAPKLLIYKASSLERGVPTRFSGSGSGTEFTLTISSLQPEDFATYHCQQYDTGATFGQGTKVEMKRTVAAPSVFIFPPSDEQLKSGTASVVCLLNNFYPREAKVQWKVDNALQSGNSQESVTEQDSKDSTYSLSSTLTLSKADYEKHKVYACEVTHQGLSSPVTKSFNRGEC

SEQ ID NO: 165 - protein, 451 aa, Artificial Sequence
  DOMAIN 1..451: note = D2-60 HC
QVQLVQSGAEVKKPGASVKVSCKASGYTFTSYGISWVRQAPGQGLEWMGWISAYNGNTNYAQKLQGRVTMTTDTSTSTAYMELRSLRSDDTAVYYCAREYSSWYSGGMDVWGQGTTVTVSSASTKGPSVFPLAPSSKSTSGGTAALGCLVKDYFPEPVTVSWNSGALTSGVHTFPAVLQSSGLYSLSSVVTVPSSSLGTQTYICNVNHKPSNTKVDKKVEPKSCDKTHTCPPCPAPEAAGGPSVFLFPPKPKDTLMISRTPEVTCVVVDVSHEDPEVKFNWYVDGVEVHNAKTKPREEQYNSTYRVVSVLTVLHQDWLNGKEYKCKVSNKALPAPIEKTISKAKGQPREPQVYTLPPSRDELTKNQVSLTCLVKGFYPSDIAVEWESNGQPENNYKTTPPVLDSDGSFFLYSKLTVDKSRWQQGNVFSCSVMHEALHNHYTQKSLSLSPGK

SEQ ID NO: 166 - protein, 214 aa, Artificial Sequence
  DOMAIN 1..214: note = D2-60 LC
DIQMTQSPSSLSASVGDRVTITCRASQGISNYLAWYQQKPGKVPKLLIYAASTLQSGVPSRFSGSGSGTDFTLTISSLQPEDVATYYCQKYDSAPFTFGQGTRLEIKRTVAAPSVFIFPPSDEQLKSGTASVVCLLNNFYPREAKVQWKVDNALQSGNSQESVTEQDSKDSTYSLSSTLTLSKADYEKHKVYACEVTHQGLSSPVTKSFNRGEC

SEQ ID NO: 167 - protein, 455 aa, Artificial Sequence
  DOMAIN 1..455: note = D3-68 HC
QVQLVQSGPEVKKPGASVKVSCKASGYTFTSYGISWVRRAPGQGLEWMGWISAYNGNTNYAQKLQGRVTMTTDTSTSTAYMELRSLRSDDTAVYYCARDLQSPTYYYGSGVIDYWGQGTLVTVSSASTKGPSVFPLAPSSKSTSGGTAALGCLVKDYFPEPVTVSWNSGALTSGVHTFPAVLQSSGLYSLSSVVTVPSSSLGTQTYICNVNHKPSNTKVDKKVEPKSCDKTHTCPPCPAPEAAGGPSVFLFPPKPKDTLMISRTPEVTCVVVDVSHEDPEVKFNWYVDGVEVHNAKTKPREEQYNSTYRVVSVLTVLHQDWLNGKEYKCKVSNKALPAPIEKTISKAKGQPREPQVYTLPPSRDELTKNQVSLTCLVKGFYPSDIAVEWESNGQPENNYKTTPPVLDSDGSFFLYSKLTVDKSRWQQGNVFSCSVMHEALHNHYTQKSLSLSPGK

SEQ ID NO: 168 - protein, 214 aa, Artificial Sequence
  DOMAIN 1..214: note = D3-68 LC
DIQLTQSPSTLSASVGDRVTISCRASRAVSPWLAWYQHRPGQAPKLLIYAASSLQSGVPSRFSGSGSGTDFTLTISSLQPEDFATYYCQQYRSYPFTFGPGTTVDIRRTVAAPSVFIFPPSDEQLKSGTASVVCLLNNFYPREAKVQWKVDNALQSGNSQESVTEQDSKDSTYSLSSTLTLSKADYEKHKVYACEVTHQGLSSPVTKSFNRGEC

SEQ ID NO: 169 - protein, 611 aa, Artificial Sequence
  DOMAIN 1..611: note = A2-22-a HC
APASSSTKKTQLQLEHLLLDLQMILNGINNYKNPKLTRMLTFKFYMPKKATELKHLQCLEEELKPLEEVLNLAQSKNFHLRPRDLISNINVIVLELKGSETTFMCEYADETATIVEFLNRWITFAQSIISTLTGGGGSGGGGSGGGGSGGGGSGGGGSQVQLVQSGAEVKKPGASVKVSCKASGYTFTSYYMHWVRQAPGQGLEWMGIINPSGGSTSYAQKFQGRVTMTRDTSTSTVYMELSSLRSEDTAVYYCAREDWMEYEYYYGMDVWGQGTLVTVSSASTKGPSVFPLAPSSKSTSGGTAALGCLVKDYFPEPVTVSWNSGALTSGVHTFPAVLQSSGLYSLSSVVTVPSSSLGTQTYICNVNHKPSNTKVDKKVEPKSCDKTHTCPPCPAPEAAGGPSVFLFPPKPKDTLMISRTPEVTCVVVDVSHEDPEVKFNWYVDGVEVHNAKTKPREEQYNSTYRVVSVLTVLHQDWLNGKEYKCKVSNKALPAPIEKTISKAKGQPREPQVYTLPPSRDELTKNQVSLTCLVKGFYPSDIAVEWESNGQPENNYKTTPPVLDSDGSFFLYSKLTVDKSRWQQGNVFSCSVMHEALHNHYTQKSLSLSPGK

SEQ ID NO: 170 - protein, 373 aa, Artificial Sequence
  DOMAIN 1..373: note = A2-22-b LC
APASSSTKKTQLQLEHLLLDLQMILNGINNYKNPKLTRMLTFKFYMPKKATELKHLQCLEEELKPLEEVLNLAQSKNFHLRPRDLISNINVIVLELKGSETTFMCEYADETATIVEFLNRWITFAQSIISTLTGGGGSGGGGSGGGGSGGGGSGGGGSEIVLTQSPGTLSLSPGERATLSCRASQSVSNNYLAWYQQKPGQAPRLLIYGASSRATGIPDRFSGSGSGTDFTLTISRLEPEDFAVYSCQQYGSSPLTFGQGTRLEIKRTVAAPSVFIFPPSDEQLKSGTASVVCLLNNFYPREAKVQWKVDNALQSGNSQESVTEQDSKDSTYSLSSTLTLSKADYEKHKVYACEVTHQGLSSPVTKSFNRGEC

SEQ ID NO: 171 - protein, 608 aa, Artificial Sequence
  DOMAIN 1..608: note = A3-21-a HC
APASSSTKKTQLQLEHLLLDLQMILNGINNYKNPKLTRMLTFKFYMPKKATELKHLQCLEEELKPLEEVLNLAQSKNFHLRPRDLISNINVIVLELKGSETTFMCEYADETATIVEFLNRWITFAQSIISTLTGGGGSGGGGSGGGGSGGGGSGGGGSEVQLLESGGGLAQPGGSLRLSCAGSGFTFSSYAMSWVRQAPGKGLEWVSGITGTGYRTYYADSVKGRFTVSRDNSRNTVYLQMNSLRAEDTAVYYCVRESGHYYGWFDSWGQGTLVTVSSASTKGPSVFPLAPSSKSTSGGTAALGCLVKDYFPEPVTVSWNSGALTSGVHTFPAVLQSSGLYSLSSVVTVPSSSLGTQTYICNVNHKPSNTKVDKKVEPKSCDKTHTCPPCPAPEAAGGPSVFLFPPKPKDTLMISRTPEVTCVVVDVSHEDPEVKFNWYVDGVEVHNAKTKPREEQYNSTYRVVSVLTVLHQDWLNGKEYKCKVSNKALPAPIEKTISKAKGQPREPQVYTLPPSRDELTKNQVSLTCLVKGFYPSDIAVEWESNGQPENNYKTTPPVLDSDGSFFLYSKLTVDKSRWQQGNVFSCSVMHEALHNHYTQKSLSLSPGK

SEQ ID NO: 172 - protein, 376 aa, Artificial Sequence
  DOMAIN 1..376: note = A3-21-b LC
APASSSTKKTQLQLEHLLLDLQMILNGINNYKNPKLTRMLTFKFYMPKKATELKHLQCLEEELKPLEEVLNLAQSKNFHLRPRDLISNINVIVLELKGSETTFMCEYADETATIVEFLNRWITFAQSIISTLTGGGGSGGGGSGGGGSGGGGSGGGGSQSALTQPPSVSGAPGQRVTISCTGSSSNIGAGYNVHWYQQVPGTVPKLLIDGKGNRPSGVPDRFSGSKSGTSASLAITGLQAEDEADYYCQSYDYMLSGSVVFGRGTKLTVLGQPKANPTVTLFPPSSEELQANKATLVCLISDFYPGAVTVAWKADGSPVKAGVETTKPSKQSNNKYAASSYLSLTPEQWKSHRSYSCQVTHEGSTVEKTVAPTECS

SEQ ID NO: 173 - protein, 610 aa, Artificial Sequence
  DOMAIN 1..610: note = B2-15-a HC
APASSSTKKTQLQLEHLLLDLQMILNGINNYKNPKLTRMLTFKFYMPKKATELKHLQCLEEELKPLEEVLNLAQSKNFHLRPRDLISNINVIVLELKGSETTFMCEYADETATIVEFLNRWITFAQSIISTLTGGGGSGGGGSGGGGSGGGGSGGGGSEVQLLESGAEVKKPGASVKVSCKASGYTFTSYYMHWVRQAPGQGLEWMGIINPSGGSTSYAQKFQGRVTMTRDTSTSTVYMELSSLRSEDTAVYYCAREGNSSGYYNAFDIWGQGTMVTVSSASTKGPSVFPLAPSSKSTSGGTAALGCLVKDYFPEPVTVSWNSGALTSGVHTFPAVLQSSGLYSLSSVVTVPSSSLGTQTYICNVNHKPSNTKVDKKVEPKSCDKTHTCPPCPAPEAAGGPSVFLFPPKPKDTLMISRTPEVTCVVVDVSHEDPEVKFNWYVDGVEVHNAKTKPREEQYNSTYRVVSVLTVLHQDWLNGKEYKCKVSNKALPAPIEKTISKAKGQPREPQVYTLPPSRDELTKNQVSLTCLVKGFYPSDIAVEWESNGQPENNYKTTPPVLDSDGSFFLYSKLTVDKSRWQQGNVFSCSVMHEALHNHYTQKSLSLSPGK

SEQ ID NO: 174 - protein, 373 aa, Artificial Sequence
  DOMAIN 1..373: note = B2-15-b LC
APASSSTKKTQLQLEHLLLDLQMILNGINNYKNPKLTRMLTFKFYMPKKATELKHLQCLEEELKPLEEVLNLAQSKNFHLRPRDLISNINVIVLELKGSETTFMCEYADETATIVEFLNRWITFAQSIISTLTGGGGSGGGGSGGGGSGGGGSGGGGSEIVLTQSPGTLSLSPGERATLSCRASQSVSSSYLAWYQQKPGQAPRLLIYGASNRATGIPDRFSGSGSGADFTLTISRLEPEDFAVYYCQQYGSSPLTFGGGTKVEIKRTVAAPSVFIFPPSDEQLKSGTASVVCLLNNFYPREAKVQWKVDNALQSGNSQESVTEQDSKDSTYSLSSTLTLSKADYEKHKVYACEVTHQGLSSPVTKSFNRGEC

SEQ ID NO: 175 - protein, 612 aa, Artificial Sequence
  DOMAIN 1..612: note = C2-53-a HC
APASSSTKKTQLQLEHLLLDLQMILNGINNYKNPKLTRMLTFKFYMPKKATELKHLQCLEEELKPLEEVLNLAQSKNFHLRPRDLISNINVIVLELKGSETTFMCEYADETATIVEFLNRWITFAQSIISTLTGGGGSGGGGSGGGGSGGGGSGGGGSEVQLVESGGGLVQPGRSLILSCAASGFTFDDYAMHWVRQAPGKGLEWVSGISWNSGSIGYADSVKGRFTISRDNAKNSLYLQMNSLRAEDTALYYCAKDQLRWGTYYYYGMDVWGQGTTVTVSSASTKGPSVFPLAPSSKSTSGGTAALGCLVKDYFPEPVTVSWNSGALTSGVHTFPAVLQSSGLYSLSSVVTVPSSSLGTQTYICNVNHKPSNTKVDKKVEPKSCDKTHTCPPCPAPEAAGGPSVFLFPPKPKDTLMISRTPEVTCVVVDVSHEDPEVKFNWYVDGVEVHNAKTKPREEQYNSTYRVVSVLTVLHQDWLNGKEYKCKVSNKALPAPIEKTISKAKGQPREPQVYTLPPSRDELTKNQVSLTCLVKGFYPSDIAVEWESNGQPENNYKTTPPVLDSDGSFFLYSKLTVDKSRWQQGNVFSCSVMHEALHNHYTQKSLSLSPGK

SEQ ID NO: 176 - protein, 371 aa, Artificial Sequence
  DOMAIN 1..371: note = C2-53-b LC
APASSSTKKTQLQLEHLLLDLQMILNGINNYKNPKLTRMLTFKFYMPKKATELKHLQCLEEELKPLEEVLNLAQSKNFHLRPRDLISNINVIVLELKGSETTFMCEYADETATIVEFLNRWITFAQSIISTLTGGGGSGGGGSGGGGSGGGGSGGGGSDIQMTQSPSTLSASVGDRVTITCRASQSVSIWVAWYQQKPGKAPKLLIYKASSLERGVPTRFSGSGSGTEFTLTISSLQPEDFATYHCQQYDTGATFGQGTKVEMKRTVAAPSVFIFPPSDEQLKSGTASVVCLLNNFYPREAKVQWKVDNALQSGNSQESVTEQDSKDSTYSLSSTLTLSKADYEKHKVYACEVTHQGLSSPVTKSFNRGEC

SEQ ID NO: 177 - protein, 609 aa, Artificial Sequence
  DOMAIN 1..609: note = D2-60-a HC
APASSSTKKTQLQLEHLLLDLQMILNGINNYKNPKLTRMLTFKFYMPKKATELKHLQCLEEELKPLEEVLNLAQSKNFHLRPRDLISNINVIVLELKGSETTFMCEYADETATIVEFLNRWITFAQSIISTLTGGGGSGGGGSGGGGSGGGGSGGGGSQVQLVQSGAEVKKPGASVKVSCKASGYTFTSYGISWVRQAPGQGLEWMGWISAYNGNTNYAQKLQGRVTMTTDTSTSTAYMELRSLRSDDTAVYYCAREYSSWYSGGMDVWGQGTTVTVSSASTKGPSVFPLAPSSKSTSGGTAALGCLVKDYFPEPVTVSWNSGALTSGVHTFPAVLQSSGLYSLSSVVTVPSSSLGTQTYICNVNHKPSNTKVDKKVEPKSCDKTHTCPPCPAPEAAGGPSVFLFPPKPKDTLMISRTPEVTCVVVDVSHEDPEVKFNWYVDGVEVHNAKTKPREEQYNSTYRVVSVLTVLHQDWLNGKEYKCKVSNKALPAPIEKTISKAKGQPREPQVYTLPPSRDELTKNQVSLTCLVKGFYPSDIAVEWESNGQPENNYKTTPPVLDSDGSFFLYSKLTVDKSRWQQGNVFSCSVMHEALHNHYTQKSLSLSPGK

SEQ ID NO: 178 - protein, 372 aa, Artificial Sequence
  DOMAIN 1..372: note = D2-60-b LC
APASSSTKKTQLQLEHLLLDLQMILNGINNYKNPKLTRMLTFKFYMPKKATELKHLQCLEEELKPLEEVLNLAQSKNFHLRPRDLISNINVIVLELKGSETTFMCEYADETATIVEFLNRWITFAQSIISTLTGGGGSGGGGSGGGGSGGGGSGGGGSDIQMTQSPSSLSASVGDRVTITCRASQGISNYLAWYQQKPGKVPKLLIYAASTLQSGVPSRFSGSGSGTDFTLTISSLQPEDVATYYCQKYDSAPFTFGQGTRLEIKRTVAAPSVFIFPPSDEQLKSGTASVVCLLNNFYPREAKVQWKVDNALQSGNSQESVTEQDSKDSTYSLSSTLTLSKADYEKHKVYACEVTHQGLSSPVTKSFNRGEC

SEQ ID NO: 179 - protein, 613 aa, Artificial Sequence
  DOMAIN 1..613: note = D3-68-a HC
APASSSTKKTQLQLEHLLLDLQMILNGINNYKNPKLTRMLTFKFYMPKKATELKHLQCLEEELKPLEEVLNLAQSKNFHLRPRDLISNINVIVLELKGSETTFMCEYADETATIVEFLNRWITFAQSIISTLTGGGGSGGGGSGGGGSGGGGSGGGGSQVQLVQSGPEVKKPGASVKVSCKASGYTFTSYGISWVRRAPGQGLEWMGWISAYNGNTNYAQKLQGRVTMTTDTSTSTAYMELRSLRSDDTAVYYCARDLQSPTYYYGSGVIDYWGQGTLVTVSSASTKGPSVFPLAPSSKSTSGGTAALGCLVKDYFPEPVTVSWNSGALTSGVHTFPAVLQSSGLYSLSSVVTVPSSSLGTQTYICNVNHKPSNTKVDKKVEPKSCDKTHTCPPCPAPEAAGGPSVFLFPPKPKDTLMISRTPEVTCVVVDVSHEDPEVKFNWYVDGVEVHNAKTKPREEQYNSTYRVVSVLTVLHQDWLNGKEYKCKVSNKALPAPIEKTISKAKGQPREPQVYTLPPSRDELTKNQVSLTCLVKGFYPSDIAVEWESNGQPENNYKTTPPVLDSDGSFFLYSKLTVDKSRWQQGNVFSCSVMHEALHNHYTQKSLSLSPGK

SEQ ID NO: 180 - protein, 372 aa, Artificial Sequence
  DOMAIN 1..372: note = D3-68-b LC
APASSSTKKTQLQLEHLLLDLQMILNGINNYKNPKLTRMLTFKFYMPKKATELKHLQCLEEELKPLEEVLNLAQSKNFHLRPRDLISNINVIVLELKGSETTFMCEYADETATIVEFLNRWITFAQSIISTLTGGGGSGGGGSGGGGSGGGGSGGGGSDIQLTQSPSTLSASVGDRVTISCRASRAVSPWLAWYQHRPGQAPKLLIYAASSLQSGVPSRFSGSGSGTDFTLTISSLQPEDFATYYCQQYRSYPFTFGPGTTVDIRRTVAAPSVFIFPPSDEQLKSGTASVVCLLNNFYPREAKVQWKVDNALQSGNSQESVTEQDSKDSTYSLSSTLTLSKADYEKHKVYACEVTHQGLSSPVTKSFNRGEC

SEQ ID NO: 181 - protein, 368 aa, Artificial Sequence
  DOMAIN 1..368: note = B2-15-b-G4S4 LC
APASSSTKKTQLQLEHLLLDLQMILNGINNYKNPKLTRMLTFKFYMPKKATELKHLQCLEEELKPLEEVLNLAQSKNFHLRPRDLISNINVIVLELKGSETTFMCEYADETATIVEFLNRWITFAQSIISTLTGGGGSGGGGSGGGGSGGGGSEIVLTQSPGTLSLSPGERATLSCRASQSVSSSYLAWYQQKPGQAPRLLIYGASNRATGIPDRFSGSGSGADFTLTISRLEPEDFAVYYCQQYGSSPLTFGGGTKVEIKRTVAAPSVFIFPPSDEQLKSGTASVVCLLNNFYPREAKVQWKVDNALQSGNSQESVTEQDSKDSTYSLSSTLTLSKADYEKHKVYACEVTHQGLSSPVTKSFNRGEC

SEQ ID NO: 182 - protein, 373 aa, Artificial Sequence
  DOMAIN 1..373: note = B2-15-b-T3E LC
APESSSTKKTQLQLEHLLLDLQMILNGINNYKNPKLTRMLTFKFYMPKKATELKHLQCLEEELKPLEEVLNLAQSKNFHLRPRDLISNINVIVLELKGSETTFMCEYADETATIVEFLNRWITFAQSIISTLTGGGGSGGGGSGGGGSGGGGSGGGGSEIVLTQSPGTLSLSPGERATLSCRASQSVSSSYLAWYQQKPGQAPRLLIYGASNRATGIPDRFSGSGSGADFTLTISRLEPEDFAVYYCQQYGSSPLTFGGGTKVEIKRTVAAPSVFIFPPSDEQLKSGTASVVCLLNNFYPREAKVQWKVDNALQSGNSQESVTEQDSKDSTYSLSSTLTLSKADYEKHKVYACEVTHQGLSSPVTKSFNRGEC

SEQ ID NO: 183 - protein, 373 aa, Artificial Sequence
  DOMAIN 1..373: note = B2-15-b-WT (IL-2) LC
APTSSSTKKTQLQLEHLLLDLQMILNGINNYKNPKLTRMLTFKFYMPKKATELKHLQCLEEELKPLEEVLNLAQSKNFHLRPRDLISNINVIVLELKGSETTFMCEYADETATIVEFLNRWITFAQSIISTLTGGGGSGGGGSGGGGSGGGGSGGGGSEIVLTQSPGTLSLSPGERATLSCRASQSVSSSYLAWYQQKPGQAPRLLIYGASNRATGIPDRFSGSGSGADFTLTISRLEPEDFAVYYCQQYGSSPLTFGGGTKVEIKRTVAAPSVFIFPPSDEQLKSGTASVVCLLNNFYPREAKVQWKVDNALQSGNSQESVTEQDSKDSTYSLSSTLTLSKADYEKHKVYACEVTHQGLSSPVTKSFNRGEC

SEQ ID NO: 184 - protein, 373 aa, Artificial Sequence
  DOMAIN 1..373: note = B2-15-b-T3Q LC
APQSSSTKKTQLQLEHLLLDLQMILNGINNYKNPKLTRMLTFKFYMPKKATELKHLQCLEEELKPLEEVLNLAQSKNFHLRPRDLISNINVIVLELKGSETTFMCEYADETATIVEFLNRWITFAQSIISTLTGGGGSGGGGSGGGGSGGGGSGGGGSEIVLTQSPGTLSLSPGERATLSCRASQSVSSSYLAWYQQKPGQAPRLLIYGASNRATGIPDRFSGSGSGADFTLTISRLEPEDFAVYYCQQYGSSPLTFGGGTKVEIKRTVAAPSVFIFPPSDEQLKSGTASVVCLLNNFYPREAKVQWKVDNALQSGNSQESVTEQDSKDSTYSLSSTLTLSKADYEKHKVYACEVTHQGLSSPVTKSFNRGEC

SEQ ID NO: 185 - protein, 370 aa, Artificial Sequence
  DOMAIN 1..370: note = B2-15-b-Del3 LC
SSSTKKTQLQLEHLLLDLQMILNGINNYKNPKLTRMLTFKFYMPKKATELKHLQCLEEELKPLEEVLNLAQSKNFHLRPRDLISNINVIVLELKGSETTFMCEYADETATIVEFLNRWITFAQSIISTLTGGGGSGGGGSGGGGSGGGGSGGGGSEIVLTQSPGTLSLSPGERATLSCRASQSVSSSYLAWYQQKPGQAPRLLIYGASNRATGIPDRFSGSGSGADFTLTISRLEPEDFAVYYCQQYGSSPLTFGGGTKVEIKRTVAAPSVFIFPPSDEQLKSGTASVVCLLNNFYPREAKVQWKVDNALQSGNSQESVTEQDSKDSTYSLSSTLTLSKADYEKHKVYACEVTHQGLSSPVTKSFNRGEC

SEQ ID NO: 186 - protein, 366 aa, Artificial Sequence
  DOMAIN 1..366: note = B2-15-b-Del7 LC
KKTQLQLEHLLLDLQMILNGINNYKNPKLTRMLTFKFYMPKKATELKHLQCLEEELKPLEEVLNLAQSKNFHLRPRDLISNINVIVLELKGSETTFMCEYADETATIVEFLNRWITFAQSIISTLTGGGGSGGGGSGGGGSGGGGSGGGGSEIVLTQSPGTLSLSPGERATLSCRASQSVSSSYLAWYQQKPGQAPRLLIYGASNRATGIPDRFSGSGSGADFTLTISRLEPEDFAVYYCQQYGSSPLTFGGGTKVEIKRTVAAPSVFIFPPSDEQLKSGTASVVCLLNNFYPREAKVQWKVDNALQSGNSQESVTEQDSKDSTYSLSSTLTLSKADYEKHKVYACEVTHQGLSSPVTKSFNRGEC

SEQ ID NO: 187 - protein, 370 aa, Artificial Sequence
  DOMAIN 1..370: note = A2-22-b-Del3 LC
SSSTKKTQLQLEHLLLDLQMILNGINNYKNPKLTRMLTFKFYMPKKATELKHLQCLEEELKPLEEVLNLAQSKNFHLRPRDLISNINVIVLELKGSETTFMCEYADETATIVEFLNRWITFAQSIISTLTGGGGSGGGGSGGGGSGGGGSGGGGSEIVLTQSPGTLSLSPGERATLSCRASQSVSNNYLAWYQQKPGQAPRLLIYGASSRATGIPDRFSGSGSGTDFTLTISRLEPEDFAVYSCQQYGSSPLTFGQGTRLEIKRTVAAPSVFIFPPSDEQLKSGTASVVCLLNNFYPREAKVQWKVDNALQSGNSQESVTEQDSKDSTYSLSSTLTLSKADYEKHKVYACEVTHQGLSSPVTKSFNRGEC

SEQ ID NO: 188 - protein, 369 aa, Artificial Sequence
  DOMAIN 1..369: note = D2-60-b-Del3 LC
SSSTKKTQLQLEHLLLDLQMILNGINNYKNPKLTRMLTFKFYMPKKATELKHLQCLEEELKPLEEVLNLAQSKNFHLRPRDLISNINVIVLELKGSETTFMCEYADETATIVEFLNRWITFAQSIISTLTGGGGSGGGGSGGGGSGGGGSGGGGSDIQMTQSPSSLSASVGDRVTITCRASQGISNYLAWYQQKPGKVPKLLIYAASTLQSGVPSRFSGSGSGTDFTLTISSLQPEDVATYYCQKYDSAPFTFGQGTRLEIKRTVAAPSVFIFPPSDEQLKSGTASVVCLLNNFYPREAKVQWKVDNALQSGNSQESVTEQDSKDSTYSLSSTLTLSKADYEKHKVYACEVTHQGLSSPVTKSFNRGEC

SEQ ID NO: 189 - protein, 372 aa, Artificial Sequence
  DOMAIN 1..372: note = D2-60-b-T3E LC
APESSSTKKTQLQLEHLLLDLQMILNGINNYKNPKLTRMLTFKFYMPKKATELKHLQCLEEELKPLEEVLNLAQSKNFHLRPRDLISNINVIVLELKGSETTFMCEYADETATIVEFLNRWITFAQSIISTLTGGGGSGGGGSGGGGSGGGGSGGGGSDIQMTQSPSSLSASVGDRVTITCRASQGISNYLAWYQQKPGKVPKLLIYAASTLQSGVPSRFSGSGSGTDFTLTISSLQPEDVATYYCQKYDSAPFTFGQGTRLEIKRTVAAPSVFIFPPSDEQLKSGTASVVCLLNNFYPREAKVQWKVDNALQSGNSQESVTEQDSKDSTYSLSSTLTLSKADYEKHKVYACEVTHQGLSSPVTKSFNRGEC

SEQ ID NO: 190 - protein, 25 aa, Artificial Sequence
  DOMAIN 1..25: note = linker
GGGGSGGGGSGGGGSGGGGSGGGGS